European Patent Application EP 4 298 897 A1, published January 3, 2024. Title: A plant belonging to genus Nicotiana and method of producing the same. Applicant: JAPAN TOBACCO INC. The sequence listing filed with the application follows.

SEQUENCE LISTING (30 sequences)

SEQ ID NO: 1 - DNA, 3138 bp, Nicotiana sylvestris
atgtcgctgttggagccggaggcgtttgatttgccggcgaaatatccgtcggaagcagctcagaggaggtggagagatgctgtttctctcgttaagaatcgccggcgtcggttccgatatgctccgaatctcgaaaaacgtgaagaagctaaagagctcatggagaaaaccagagaaaagattcgagttggtttcatggcttatatggcagcactcaagttcattgatgctggtgatcatggtaggccttctgaccaggtcagagaagatataggggctgaactggcaaaagacttgccagaaggagctcgaaatgctggttttggaattaaccctgataaacttgcatctatagttggttcctatgatataaaaaccttaaataaacttggaggtgtcgaagggcttgcaggtaaattgaaagtctcatcaaacgaaggagtcaaatctagtgatgtacctatgagacaaaatatatatggatcaaacaaattcactgagaaaccttttagaagtttttggacatttgtgtgggaggctctgcatgatttaactctcgtcatcctgatagtttgtgctgttgtttccattggcgtcggacttgctactgaaggttggccaaaaggaacatatgatggtttaggaattctactcagcatattcttggtagtctttgttactgcagttagtgactataggcagtcgttgcagttcagggatttggataaggagaagaaaaagatatccatccaggtcacaagagatggatcaaggcagaaggtttccatttatgacttggtggttggtgatgtagttcacttatctattggagatcttgttccggctgatggaatattcatatcaggatatagtttgctaattgatcaatcgagcttgtctggtgagagtgtaccagtaagcatatatgaaaaaagaccttttcttttatcaggaactaaagtacaagatggttcagctaagatgttagtgaccactgttggtatgagaactgaatggggtaagcttatggaaactcttagcgagggaggagaagatgagactcctctgcaagttaagctgaatggtgttgccactattattggaaagatagggctggggtttgctgtggtgacatttcttgtgttaatagtcagatttctggtggataaagcaaatcaccatcaattcaccgaatggtcgtccagtgatgcattaactcttctaaattactttgccactgctgtaactataattgttgttgcagttcctgaaggactacctctggctgtcacattgagccttgcatttgcaatgaaaaagttaatggacaataaagcgttagtgaggcatctttctgcttgtgagacaatgggttcagcatcttgcatctgcacggataagacaggaacactaacaacaaaccatatggtagtaaataaaatatggatttgcggaaaggctaaaaaggtagaaaatgatacaggtggagatgcaataacggacatatcagaaagtgcactggactttcttttgcaggcaatatttcataatacaggagctgaggtggttaaaggcaaggatggaaagaaatctgttctgggtacacccacagaatctgcaatattggaatacggattacttcttggtgatattgatgataaaaaaagggattgtaatatgctgaaggttgaacctttcaattcagcaaagaaaagaatgtcagtgcttgttgctcttcctgacggcaacacccgtgcgttctgcaagggtgcatctgagatagttttgaaaatgtgtgacaggtttattgattccaatggtgaaattgttgatatgtcagaagaacaggttacaaacatcatggatgtcattaaggaatttgctgatgaagccttgcgtactctttgcttggcgttcaaggatattgaagatggttatcaagaaaataatatccccgatcatggctacacattggttgcagtcgttggaatcaaagatccagttcgccctggggttaaagaggcggttaaaacttgtttagctgctggaattactgtaaggatggtcacaggggacaatattaatacggctatagccattgctaaagaatgtggtatactaactgccgatggtttggccattgaaggcccagaatttcgcaacaaaagtcctgatgaaatgagacaaatacttcctagaattcaggttatggctcgatcatcccctacagacaagcatgtgctggtaaagaatttaagaggcatgtttagagaagttgtcgcagttactggtgatggcacaaatgatgcccctgctctgcatgagtcagatattggactggccatgggtatagcaggaacagaggttgcaaaagaaagtgctgatattatagtgcttgatgacaacttcaggacaattgtgaatgtggctaaatggggccgttctgtatatataaacattcaaaaattcgtgcaatttcagttgactgtcaatgttgtggctctgatgatcaattttatttctgcatgcgcctcaggatctgctcctctcactgctgttcagctgctttgggtcaaccttatcatggatactttaggtgcattggcactggccactgaaccaccccatgatggactaatgagtcggcctcctgttggaagggatgtgagtttcattacaaagacaatgtggagaaacataataggacacagtatctaccagctggctatactcttaaccttcaactttgccggaaagcagattttgagacttgaaggttcagatgctacaaaaatccagaataccttcatttttaacacctttgtgttttgtcaggtgttcaacgaaataaacagtcgtgatatgcagaagataaacattttccgtggcatttttagcagctggattttcttaggagtcatggttgctacagttgttttccaagttatcatcgtcgagttcttaggcacttttgccagcactacaccacttagctggcaactatggctgatcagtgtcttgattggtgctgcaagcttgatcgttgctattattttgaagttgatccctgtcgaaaaggagacttctaagcaccatgacggctatgatctgctaccaagtggtccagaacttgcctag

SEQ ID NO: 2 - protein, 1045 aa, Nicotiana sylvestris
MSLLEPEAFDLPAKYPSEAAQRRWRDAVSLVKNRRRRFRYAPNLEKREEAKELMEKTREKIRVGFMAYMAALKFIDAGDHGRPSDQVREDIGAELAKDLPEGARNAGFGINPDKLASIVGSYDIKTLNKLGGVEGLAGKLKVSSNEGVKSSDVPMRQNIYGSNKFTEKPFRSFWTFVWEALHDLTLVILIVCAVVSIGVGLATEGWPKGTYDGLGILLSIFLVVFVTAVSDYRQSLQFRDLDKEKKKISIQVTRDGSRQKVSIYDLVVGDVVHLSIGDLVPADGIFISGYSLLIDQSSLSGESVPVSIYEKRPFLLSGTKVQDGSAKMLVTTVGMRTEWGKLMETLSEGGEDETPLQVKLNGVATIIGKIGLGFAVVTFLVLIVRFLVDKANHHQFTEWSSSDALTLLNYFATAVTIIVVAVPEGLPLAVTLSLAFAMKKLMDNKALVRHLSACETMGSASCICTDKTGTLTTNHMVVNKIWICGKAKKVENDTGGDAITDISESALDFLLQAIFHNTGAEVVKGKDGKKSVLGTPTESAILEYGLLLGDIDDKKRDCNMLKVEPFNSAKKRMSVLVALPDGNTRAFCKGASEIVLKMCDRFIDSNGEIVDMSEEQVTNIMDVIKEFADEALRTLCLAFKDIEDGYQENNIPDHGYTLVAVVGIKDPVRPGVKEAVKTCLAAGITVRMVTGDNINTAIAIAKECGILTADGLAIEGPEFRNKSPDEMRQILPRIQVMARSSPTDKHVLVKNLRGMFREVVAVTGDGTNDAPALHESDIGLAMGIAGTEVAKESADIIVLDDNFRTIVNVAKWGRSVYINIQKFVQFQLTVNVVALMINFISACASGSAPLTAVQLLWVNLIMDTLGALALATEPPHDGLMSRPPVGRDVSFITKTMWRNIIGHSIYQLAILLTFNFAGKQILRLEGSDATKIQNTFIFNTFVFCQVFNEINSRDMQKINIFRGIFSSWIFLGVMVATVVFQVIIVEFLGTFASTTPLSWQLWLISVLIGAASLIVAIILKLIPVEKETSKHHDGYDLLPSGPELA

SEQ ID NO: 3 - DNA, 3138 bp, Nicotiana tabacum
atgtcgctgttggagccggaggcgtttgatttgccggcgaaatatccgtcggaagcagctcagaggaggtggagagatgctgtttctctcgttaagaatcgccggcgtcggttcagatatgctccgaatctcgaaaaacgtgaagaagctaaagagctcatggagaaaaccagagaaaagattcgagttggtttcatggcttatatggcagcactcaagttcattgatgctggtgatcatggtaggccttctgaccaggtcagagaagatataggggctgaactggcaaaagacttgccagaaggagctcgaaatgctggttttggaattaaccctgataaacttgcatctatagttggttcctatgatataaaaaccttaaataaacttggaggtgtcgaagggcttgcaggtaaattgaaagtctcatcaaacgaaggagtcaaatctagtgatgtacctatgagacaaaatatatatggatcaaacaaattcactgagaaaccttttagaagtttttggacatttgtgtgggaggctctgcatgatttaactctcgtcatcctgatagtttgtgctgttgtttccattggcgtcggacttgctactgaaggttggccaaaaggaacatatgatggtttaggaattctactcagcatattcttggtagtctttgttactgcagttagtgactataggcagtcgttgcagttcagggatttggataaggagaagaaaaagatatccatccaggtcacaagagatggatcaaggcagaaggtttccatttatgacttggtggttggtgatgtagttcacttatctattggagatcttgttccggctgatggaatattcatatcaggatatagtttgctaattgatcaatcgagcttgtctggtgagagtgtaccagtaagcatatatgaaaaaagaccttttcttttatcaggaactaaagtacaagatggttcagctaagatgttagtgaccactgttggtatgagaactgaatggggtaagcttatggaaactcttagcgagggaggagaagatgagactcctctgcaagttaagctgaatggtgttgccactattattggaaagatagggctggggtttgctgtggtgacatttcttgtgttaatagtcagatttctggtggataaagcaaatcaccatcaattcaccgaatggtcgtccagtgatgcattaactcttctaaattactttgccactgctgtaactataattgttgttgcagttcctgaaggactacctctggctgtcacattgagccttgcatttgcaatgaaaaagttaatggacaataaagcgttagtgaggcatctttctgcttgtgagacaatgggttcagcatcttgcatctgcacggataagacaggaacactaacaacaaaccatatggtagtaaataaaatatggatttgcggaaaggctaaaaaggtagaaaatgatacaggtggagatgcaataacggacatatcagaaagtgcactggactttcttttgcaggcaatatttcataatacaggagctgaggtggttaaaggcaaggatggaaagaaatctgttctgggtacacccacagaatctgcaatattggaatacggattacttcttggtgatattgatgataaaaaaagggattgtaatatgctgaaggttgaacctttcaattcagcaaagaaaagaatgtcagtgcttgttgctcttcctgacggcaacacccgtgcgttctgcaagggtgcatctgagatagttttgaaaatgtgtgacaggtttattgattccaatggtgaaattgttgatatgtcagaagaacaggttacaaacatcatggatgtcattaaggaatttgctgatgaagccttgcgtactctttgcttggcgttcaaggatattgaagatggttatcaagaaaataatatccccgatcatggctacacattggttgcagtcgttggaatcaaagatccagttcgccctggggttaaagaggcggttaaaacttgtttagctgctggaattactgtaaggatggtcacaggggacaatattaatacggctatagccattgctaaagaatgtggtatactaactgccgatggtttggccattgaaggcccagaatttcgcaacaaaagtcctgatgaaatgagacaaatacttcctagaattcaggttatggctcgatcatcccctacagacaagcatgtgctggtaaagaatttaagaggcatgtttagagaagttgtcgcagttactggtgatggcacaaatgatgcccctgctctgcatgagtcagatattggactggccatgggtatagcaggaacagaggttgcaaaagaaagtgctgatattatagtgcttgatgacaacttcaggacaattgtgaatgtggctaaatggggccgttctgtatatataaacattcaaaaattcgtgcaatttcagttgactgtcaatgttgtggctctgatgatcaattttatttctgcatgcgcctcaggatctgctcctctcactgctgttcagctgctttgggtcaaccttatcatggatactttaggtgcattggcactggccactgaaccaccccatgatggactaatgagtcggcctcctgttggaagggatgtgagtttcattacaaagacaatgtggagaaacataataggacacagtatctaccagctggctatactcttaaccttcaactttgccggaaagcagattttgagacttgaaggttcagatgctacaaaaatccagaataccttcatttttaacacctttgtgttttgtcaggtgttcaacgaaataaacagtcgtgatatgcagaagataaacattttccgtggcatttttagcagctggattttcttaggagtcatggttgctacagttgttttccaagttatcatcgtcgagttcttaggcacttttgccagcactacaccacttagctggcaactatggctgatcagtgtcttgattggtgctgcaagcttgatcgttgctattattttgaagttgatccctgtcgaaaaggagacttctaagcaccatgacggctatgatctgctaccaagtggtccagaacttgcctag

SEQ ID NO: 4 - protein, 1045 aa, Nicotiana tabacum; identical to SEQ ID NO: 2

SEQ ID NO: 5 - DNA, 3138 bp, Nicotiana tabacum
atgtcgctgttggagccggaagcgtttgatttgccggcgaaatatccgtcggaagcagctcagaggaggtggagagatgctgtttctctcgttaagaatcgccggcgtcggttccgatatgctccgaatctcgaaaaacgtgaagaagctaaagagcttatggagaaaaccagagaaaagattcgagttggtttcatggcttatatggcagcactcaagttcattgatgctggtgatcatggtaggccttctgaccaggtcagagaagatataggggctgaactggcaaaagacttgccagaagaagctcgagatgctggttttggaattaaccctgataaacttgcatctatagttggttcctatgatataaaaaccttaaagaaacttggaggtgttgaagggcttgcaggtaaattgagagtcacatcaaacgaaggagtcaaatctagtgatgtacctgtaagacaaaatatatatggatcaaacgaattcaccgagaaaccttttagaagtttttggacatttgtgtgggaggctctgcatgatttaactctcgtcatcctgatagtttgtgctgttgtttccattggtgtcggacttgctactgaagggtggccaaaaggaacatatgatggtttaggaattctactcagcatattcttggtagtctttgttactgcagttagtgactataggcagtcgttgcagttcagggatttggataaggagaagaaaaagatatccatccaggtcacaagagatggatcaaggcagaaggtttccatttatgacttggtggttggtgatgtagttcacttatctattggagatcttgttccggctgatggaatattcatatcaggatatagcttgctaattgatcaatcgagtttgtctggtgagagtgtaccagtaagcatatatgaaaaaagaccctttcttctatcaggaaccaaagtacaagatggttcagctaagatgctagtgaccactgttggtatgagaactgaatggggtaagcttatggaaactcttagcgagggaggagaagatgagactcctctacaagttaagctgaatggtgttgccactattattggaaagatagggctgggatttgctgtggtgacatttcttgtgttaatagtcagatttatggtggataaagctactcaccatcaattcaccaaatggtcttccagtgatgcattaactcttctaaattactttgccaccgctgtaactataatcgttgttgcagttcctgaaggactacctctggctgtcacattgagccttgcatttgcaatgaaaaagttaatggataataaagcattagtgaggcatctttctgcttgtgagacaatgggttcagcatcttgcatctgcacggataagacaggaacactaacaacaaaccatatggtagtaaataaaatatggatttgcggaaaggctaaaaaggtagaaaatggtgcaggtggagatgcaataacggatatatcagaaagtgcactggactttcttttgcaggcaatatttcataatacaggagctgaggtggttaaagacaaggatggaaagaaatatgttctgggtacacccacagaatctgcaatattagaatacggattacttcttggtgatattgatgataaaaaaagggattgtaatatgctgaaggttgaaccgttcaattcagcaaagaaaagaatgtcagtgcttgttgctcttcctgatggcaatacccgtgctttctgcaagggtgcatctgagatagttttgaaaatgtgtgacaggtttattgattccaatggtgaaattgttgatatgtcagaagaacatgttacaaacatcatgggtgtcattaaggaatttgctgatggcgccttgcgtactctttgcttggctttcaaggatatcgaagatggttatcaagaaaataatatccccgataatggctacacattggttgcagtagttggaatcaaagatccagttcgccctggggttaaagaggcagttaaaacttgtttagctgctggaattactgtaaggatggtcacaggggacaatattaatacggccatagctattgctaaagaatgtggtatactaactgctgatggtttggccattgaaggcccagaatttcgcaacaaaagtcctgatgaaatgaggcaaatacttcctagaattcaggttatggctcgatcatcccctacagacaagcatgtgctggtaaagaatttaagaggcatgtttagagaagttgtcgcagttactggtgatggcacaaatgatgcccctgctctgcatgagtcagatattggactggccatgggtatagcaggaacagaggttgcaaaagaaagtgctgatattatagtgcttgatgacaacttcaggacaattgtgaatgtggctaaatggggccgttctgtatatataaacattcaaaaattcgtgcaattccagttgactgtcaatgttgtggctctgatgatcaattttatttctgcatgcgcctcaggatctgctcctctcactgctgttcagctgctttgggtcaaccttatcatggatactttaggtgcattggcactggccactgaaccgccccatgaaggactaatgagtcggcctcctgttggaagggatgtgagtttcattacaaagacaatgtggagaaacataataggacacagtatctaccagctggctatactcttaaccttcaacttcgccggaaagcagattttgaaacttgaaggttcagatgctacaaaaatccagaataccttcatttttaacacctttgtgttttgtcaggtgttcaacgaaataaacagtcgtgatatgcagaagataaacattttccgtggcatttttagcagctggattttcttaggagtcatgtttgctacagttgttttccaagttatcatcgtcgagttcttaggcacttttgccagcactacaccactaagctggcaactatggctgatcagtgtcttgattggtgctgcaagcttgatcattgctgttattttgaagttgatccctgtcgaaaaggagacttctaagcaccatgacggctatgatctaataccaagtggtccagaacttgcctag

SEQ ID NO: 6 - protein, 1045 aa, Nicotiana tabacum
MSLLEPEAFDLPAKYPSEAAQRRWRDAVSLVKNRRRRFRYAPNLEKREEAKELMEKTREKIRVGFMAYMAALKFIDAGDHGRPSDQVREDIGAELAKDLPEEARDAGFGINPDKLASIVGSYDIKTLKKLGGVEGLAGKLRVTSNEGVKSSDVPVRQNIYGSNEFTEKPFRSFWTFVWEALHDLTLVILIVCAVVSIGVGLATEGWPKGTYDGLGILLSIFLVVFVTAVSDYRQSLQFRDLDKEKKKISIQVTRDGSRQKVSIYDLVVGDVVHLSIGDLVPADGIFISGYSLLIDQSSLSGESVPVSIYEKRPFLLSGTKVQDGSAKMLVTTVGMRTEWGKLMETLSEGGEDETPLQVKLNGVATIIGKIGLGFAVVTFLVLIVRFMVDKATHHQFTKWSSSDALTLLNYFATAVTIIVVAVPEGLPLAVTLSLAFAMKKLMDNKALVRHLSACETMGSASCICTDKTGTLTTNHMVVNKIWICGKAKKVENGAGGDAITDISESALDFLLQAIFHNTGAEVVKDKDGKKYVLGTPTESAILEYGLLLGDIDDKKRDCNMLKVEPFNSAKKRMSVLVALPDGNTRAFCKGASEIVLKMCDRFIDSNGEIVDMSEEHVTNIMGVIKEFADGALRTLCLAFKDIEDGYQENNIPDNGYTLVAVVGIKDPVRPGVKEAVKTCLAAGITVRMVTGDNINTAIAIAKECGILTADGLAIEGPEFRNKSPDEMRQILPRIQVMARSSPTDKHVLVKNLRGMFREVVAVTGDGTNDAPALHESDIGLAMGIAGTEVAKESADIIVLDDNFRTIVNVAKWGRSVYINIQKFVQFQLTVNVVALMINFISACASGSAPLTAVQLLWVNLIMDTLGALALATEPPHEGLMSRPPVGRDVSFITKTMWRNIIGHSIYQLAILLTFNFAGKQILKLEGSDATKIQNTFIFNTFVFCQVFNEINSRDMQKINIFRGIFSSWIFLGVMFATVVFQVIIVEFLGTFASTTPLSWQLWLISVLIGAASLIIAVILKLIPVEKETSKHHDGYDLIPSGPELA

SEQ ID NO: 7 - DNA, 25 bp, Artificial Sequence
  Synthetic Primer
cacctgatgctggtgatcatggtag

SEQ ID NO: 8 - DNA, 22 bp, Artificial Sequence
  Synthetic Primer
atttacctgcaagcccttcgac

SEQ ID NO: 9 - DNA, 24 bp, Artificial Sequence
  Artificial Sequence
cacctgtttccatcaatgcctgag

SEQ ID NO: 10 - DNA, 22 bp, Artificial Sequence
  Synthetic Primer
tcatacatacaaggagccaaag

SEQ ID NO: 11 - DNA, 25 bp, Artificial Sequence
  Synthetic Primer
aatgtgtgacaggtttattgattcc

SEQ ID NO: 12 - DNA, 23 bp, Artificial Sequence
  Synthetic Primer
atatccttgaacgccaagcaaag

SEQ ID NO: 13 - DNA, 30 bp, Artificial Sequence
  Probe
acgcaaggcttcatcagcaaattccttaat

SEQ ID NO: 14 - DNA, 26 bp, Artificial Sequence
  Synthetic Primer
aattgttcctctgacagaaaatagaa

SEQ ID NO: 15 - DNA, 22 bp, Artificial Sequence
  Synthetic Primer
ccatcctcaaagtccttgaagg

SEQ ID NO: 16 - DNA, 28 bp, Artificial Sequence
  Probe
cacacaaagagtacgcaaggcttcgcca

SEQ ID NO: 17 - DNA, 25 bp, Artificial Sequence
  Synthetic Primer
gctagacagtgtaatcttgacaagg

SEQ ID NO: 18 - DNA, 26 bp, Artificial Sequence
  Synthetic Primer
cgagactcgatctccataatcttaga

SEQ ID NO: 19 - DNA, 29 bp, Artificial Sequence
  Probe
tttcctaccacaaggtcacgctctttggc

SEQ ID NO: 20 - DNA, 20 bp, Artificial Sequence
  Synthetic Primer
ctaagggtgctgccagcttt

SEQ ID NO: 21 - DNA, 22 bp, Artificial Sequence
  Synthetic Primer
gtcaagcactggagcatatcca

SEQ ID NO: 22 - DNA, 26 bp, Artificial Sequence
  Probe
atcatgaaccatccaggacagattgg

SEQ ID NO: 23 - DNA, 30 bp, Artificial Sequence
  Primer
taagagacagtggcgttcaaggatattgaa

SEQ ID NO: 24 - DNA, 30 bp, Artificial Sequence
  Primer
taagagacagttctttagcaatggctatag

SEQ ID NO: 25 - DNA, 30 bp, Artificial Sequence
  Primer
taagagacagagtgatgtacctatgagaca

SEQ ID NO: 26 - DNA, 30 bp, Artificial Sequence
  Primer
taagagacaggtactttagttcctgataaa

SEQ ID NO: 27 - DNA, 30 bp, Artificial Sequence
  Primer
taagagacagataaaatttccggctaacat

SEQ ID NO: 28 - DNA, 30 bp, Artificial Sequence
  Primer
taagagacaggaggtgaaaacatactctgg

SEQ ID NO: 29 - DNA, 30 bp, Artificial Sequence
  Primer
taagagacagtctagtgatgtacctgtaag

SEQ ID NO: 30 - DNA, 30 bp, Artificial Sequence
  Primer
taagagacaggtactttggttcctgataga